European Patent Application EP 4 276 466 A1, published November 15, 2023. Title: ANTIBODY SPECIFICALLY BINDING WITH PD-L1 AND ANTIGEN-BINDING FRAGMENT OF ANIIBODY. Applicant: BEIJING HANMI PHARMACEUTICAL CO., LTD. The sequence listing filed with the application follows.

SEQUENCE LISTING (61 sequences)

SEQ ID NO: 1 - DNA, 36 bp, Artificial
  PCR primer
gaggtgaagctgcaggagtcaggacctagcctggtg

SEQ ID NO: 2 - DNA, 22 bp, Artificial
  PCR primer
aggtsmaactgcagsagtcwgg

SEQ ID NO: 3 - DNA, 22 bp, Artificial
  PCR primer
aggtsmagctgcagsagtcwgg

SEQ ID NO: 4 - DNA, 22 bp, Artificial
  PCR primer
aggtscagctgcagsagtcwgg

SEQ ID NO: 5 - DNA, 38 bp, Artificial
  PCR primer
ccaggggccagtggatagacaagcttgggtgtcgtttt

SEQ ID NO: 6 - DNA, 27 bp, Artificial
  PCR primer
atagacagatgggggtgtcgttttggc

SEQ ID NO: 7 - DNA, 23 bp, Artificial
  PCR primer
cttgaccaggcatcctagagtca

SEQ ID NO: 8 - DNA, 24 bp, Artificial
  PCR primer
aggggccagtggatagactgatgg

SEQ ID NO: 9 - DNA, 24 bp, Artificial
  PCR primer
agggaccaagggatagacagatgg

SEQ ID NO: 10 - DNA, 20 bp, Artificial
  PCR primer
  misc_feature (6)..(6): n is a, c, g or t
sargtnmagctgsagsagtc

SEQ ID NO: 11 - DNA, 23 bp, Artificial
  PCR primer
  misc_feature (6)..(6): n is a, c, g or t
sargtnmagctgsagsagtcwgg

SEQ ID NO: 12 - DNA, 32 bp, Artificial
  PCR primer
ggtgatatcgtgatracmcargatgaactctc

SEQ ID NO: 13 - DNA, 32 bp, Artificial
  PCR primer
ggtgatatcwtgmtgacccaawctccactctc

SEQ ID NO: 14 - DNA, 32 bp, Artificial
  PCR primer
ggtgatatcgtkctcacycartctccagcaat

SEQ ID NO: 15 - DNA, 32 bp, Artificial
  PCR primer
gggaagatggatccagttggtgcagcatcagc

SEQ ID NO: 16 - DNA, 21 bp, Artificial
  PCR primer
ggatacagttggtgcagcatc

SEQ ID NO: 17 - DNA, 24 bp, Artificial
  PCR primer
gayattgtgmtsacmcarwctmca

SEQ ID NO: 18 - protein, 107 aa, Artificial
  Antibody light chain variable region
DIVMTQSHKVMSTSVGDRVTITCKASQDVHTAVAWIHQKPGQSPKLLIYSASNRYTGVPDRFTGSGSGTDFTFTISSVQAEDLAVYYCQQHYITPLTFGAGTTLELK

SEQ ID NO: 19 - protein, 117 aa, Artificial
  Antibody heavy chain variable region
EVQLQQSGAELVKPGASVKLSCTASGFNIEDTYIHWVMQRPEQGLEWIGRIDPANGNTKYDPKFQGKATITADTSSNTAYLQLSSLTSEDTAVYYCGRGLGAWFAYWGQGTLVTVSA

SEQ ID NO: 20 - protein, 11 aa, Artificial
  LCDR1
KASQDVHTAVA

SEQ ID NO: 21 - protein, 7 aa, Artificial
  LCDR2
SASNRYT

SEQ ID NO: 22 - protein, 9 aa, Artificial
  LCDR3
QQHYITPLT

SEQ ID NO: 23 - protein, 10 aa, Artificial
  HCDR1
GFNIEDTYIH

SEQ ID NO: 24 - protein, 17 aa, Artificial
  HCDR2
RIDPANGNTKYDPKFQG

SEQ ID NO: 25 - protein, 8 aa, Artificial
  HCDR3
GLGAWFAY

SEQ ID NO: 26 - protein, 107 aa, Artificial [sequence omitted]

SEQ ID NO: 27 - protein, 330 aa, Artificial [sequence omitted]

SEQ ID NO: 28 - protein, 95 aa, Artificial
  Template for light chain variable region
DIQMTQSPSSLSASVGDRVTITCQASQDISNYLNWYQQKPGKAPKLLIYDASNLETGVPSRFSGSGSGTDFTFTISSLQPEDIATYYCQQYDNLP

SEQ ID NO: 29 - protein, 98 aa, Artificial
  Template for heavy chain variable region
QVQLVQSGAEVKKPGSSVKVSCKASGGTFSSYAISWVRQAPGQGLEWMGGIIPIFGTANYAQKFQGRVTITADKSTSTAYMELSSLRSEDTAVYYCAR

SEQ ID NO: 30 - protein, 117 aa, Artificial
  Heavy chain variable region
QVQLVQSGAEVKKPGSSVKVSCTASGFNIEDTYIHWVRQAPGQGLEWMGRIDPANGNTKYDPKFQGRVTITADESTSTAYMELSSLRSEDTAVYYCGRGLGAWFAYWGQGTLVTVSS

SEQ ID NO: 31 - protein, 117 aa, Artificial
  Heavy chain variable region
QVQLVQSGAEVKKPGSSVKVSCTASGFNIEDTYIHWVRQAPGQGLEWMGRIDPANGNTKYDPKFQGRATITADESTSTAYMELSSLRSEDTAVYYCGRGLGAWFAYWGQGTLVTVSS

SEQ ID NO: 32 - protein, 117 aa, Artificial
  Heavy chain variable region
QVQLVQSGAEVKKPGSSVKVSCTASGFNIEDTYIHWVRQAPGQGLEWMGRIDPANGNTKYDPKFQGRVTITADTSTSTAYMELSSLRSEDTAVYYCGRGLGAWFAYWGQGTLVTVSS

SEQ ID NO: 33 - protein, 117 aa, Artificial
  Heavy chain variable region
QVQLVQSGAEVKKPGSSVKVSCTASGFNIEDTYIHWVRQAPGQGLEWMGRIDPANGNTKYDPKFQGRVTITADESTNTAYMELSSLRSEDTAVYYCGRGLGAWFAYWGQGTLVTVSS

SEQ ID NO: 34 - protein, 117 aa, Artificial
  Heavy chain variable region
QVQLVQSGAEVKKPGSSVKVSCTASGFNIEDTYIHWVRQAPGQGLEWMGRIDPANGNTKYDPKFQGRATITADTSTSTAYMELSSLRSEDTAVYYCGRGLGAWFAYWGQGTLVTVSS

SEQ ID NO: 35 - protein, 117 aa, Artificial
  Heavy chain variable region
QVQLVQSGAEVKKPGSSVKVSCTASGFNIEDTYIHWVRQAPGQGLEWMGRIDPANGNTKYDPKFQGRATITADESTNTAYMELSSLRSEDTAVYYCGRGLGAWFAYWGQGTLVTVSS

SEQ ID NO: 36 - protein, 117 aa, Artificial
  Heavy chain variable region
QVQLVQSGAEVKKPGSSVKVSCTASGFNIEDTYIHWVRQAPGQGLEWMGRIDPANGNTKYDPKFQGRVTITADTSTNTAYMELSSLRSEDTAVYYCGRGLGAWFAYWGQGTLVTVSS

SEQ ID NO: 37 - protein, 117 aa, Artificial
  Heavy chain variable region
QVQLVQSGAEVKKPGSSVKVSCTASGFNIEDTYIHWVRQAPGQGLEWMGRIDPANGNTKYDPKFQGRATITADTSTNTAYMELSSLRSEDTAVYYCGRGLGAWFAYWGQGTLVTVSS

SEQ ID NO: 38 - protein, 107 aa, Artificial
  Light chain variable region
DIQMTQSPSSLSASVGDRVTITCKASQDVHTAVAWYQQKPGKAPKLLIYSASNRYTGVPSRFSGSGSGTDFTFTISSLQPEDIATYYCQQHYITPLTFGQGTKLEIK

SEQ ID NO: 39 - protein, 107 aa, Artificial
  Light chain variable region
DIQMTQSPSSLSASVGDRVTITCKASQDVHTAVAWIHQKPGKAPKLLIYSASNRYTGVPSRFSGSGSGTDFTFTISSLQPEDIATYYCQQHYITPLTFGQGTKLEIK

SEQ ID NO: 40 - protein, 117 aa, Artificial
  Heavy chain variable region
EVQLVQSGAEVKKPGSSVKVSCKASGFNIEDTYIHWVRQAPGQGLEWMGRIDPANGNTKYDPKFQGRVTITADESTNTAYMELSSLRSEDTAVYYCGRGLGAWFAYWGQGTLVTVSS

SEQ ID NO: 41 - protein, 117 aa, Artificial
  Heavy chain variable region
EVQLVQSGAEVKKPGSSVKVSCKASGFNIEDTYIHWVRQAPGQGLEWMGRIDPANGNTKYDPKFQGRVTITADTSTNTAYMELSSLRSEDTAVYYCGRGLGAWFAYWGQGTLVTVSS

SEQ ID NO: 42 - protein, 117 aa, Artificial
  Heavy chain variable region
EVQLVQSGAEVKKPGSSVKVSCKASGFNIEDTYIHWVRQAPGQGLEWIGRIDPANGNTKYDPKFQGRATITADESTNTAYMELSSLRSEDTAVYYCGRGLGAWFAYWGQGTLVTVSS

SEQ ID NO: 43 - protein, 117 aa, Artificial
  Heavy chain variable region
EVQLVQSGAEVKKPGSSVKVSCKASGFNIEDTYIHWVRQAPGQGLEWIGRIDPANGNTKYDPKFQGRATITADTSTNTAYMELSSLRSEDTAVYYCGRGLGAWFAYWGQGTLVTVSS

SEQ ID NO: 44 - protein, 107 aa, Artificial
  Light chain variable region
DIQMTQSPSSLSASVGDRVTITCKASQDVHTAVAWIQQKPGKSPKLLIYSASNRYTGVPSRFSGSGSGTDFTFTISSLQPEDIATYYCQQHYITPLTFGQGTKLEIK

SEQ ID NO: 45 - protein, 17 aa, Artificial
  Muated HCDR2
RIDPAQGNTKYDPKFQG

SEQ ID NO: 46 - protein, 17 aa, Artificial
  Mutated HCDR2
RIDPASGNTKYDPKFQG

SEQ ID NO: 47 - protein, 17 aa, Artificial
  Mutated HCDR2
RIDPANANTKYDPKFQG

SEQ ID NO: 48 - protein, 117 aa, Artificial
  Mutated heavy chain variable region
QVQLVQSGAEVKKPGSSVKVSCTASGFNIEDTYIHWVRQAPGQGLEWMGRIDPAQGNTKYDPKFQGRVTITADTSTNTAYMELSSLRSEDTAVYYCGRGLGAWFAYWGQGTLVTVSS

SEQ ID NO: 49 - protein, 117 aa, Artificial
  Mutated heavy chain variable region
QVQLVQSGAEVKKPGSSVKVSCTASGFNIEDTYIHWVRQAPGQGLEWMGRIDPASGNTKYDPKFQGRVTITADTSTNTAYMELSSLRSEDTAVYYCGRGLGAWFAYWGQGTLVTVSS

SEQ ID NO: 50 - protein, 117 aa, Artificial
  Mutated heavy chain variable region
QVQLVQSGAEVKKPGSSVKVSCTASGFNIEDTYIHWVRQAPGQGLEWMGRIDPANANTKYDPKFQGRVTITADTSTNTAYMELSSLRSEDTAVYYCGRGLGAWFAYWGQGTLVTVSS

SEQ ID NO: 51 - protein, 117 aa, Artificial
  Mutated heavy chain variable region
EVQLVQSGAEVKKPGSSVKVSCKASGFNIEDTYIHWVRQAPGQGLEWMGRIDPAQGNTKYDPKFQGRVTITADTSTNTAYMELSSLRSEDTAVYYCGRGLGAWFAYWGQGTLVTVSS

SEQ ID NO: 52 - protein, 117 aa, Artificial
  Mutated heavy chain variable region
EVQLVQSGAEVKKPGSSVKVSCKASGFNIEDTYIHWVRQAPGQGLEWMGRIDPASGNTKYDPKFQGRVTITADTSTNTAYMELSSLRSEDTAVYYCGRGLGAWFAYWGQGTLVTVSS

SEQ ID NO: 53 - protein, 117 aa, Artificial
  Mutated heavy chain variable region
EVQLVQSGAEVKKPGSSVKVSCKASGFNIEDTYIHWVRQAPGQGLEWMGRIDPANANTKYDPKFQGRVTITADTSTNTAYMELSSLRSEDTAVYYCGRGLGAWFAYWGQGTLVTVSS

SEQ ID NO: 54 - protein, 23 aa, Artificial
DIQMTQSPSSLSASVGDRVTITC

SEQ ID NO: 55 - protein, 15 aa, Artificial
WYQQKPGKAPKLLIY

SEQ ID NO: 56 - protein, 32 aa, Artificial
  FR-L3
GVPSRFSGSGSGTDFTFTISSLQPEDIATYYC

SEQ ID NO: 57 - protein, 10 aa, Artificial
  FR-L4
FGQGTKLEIK

SEQ ID NO: 58 - protein, 25 aa, Artificial [sequence omitted]

SEQ ID NO: 59 - protein, 14 aa, Artificial
  FR-H2
WVRQAPGQGLEWMG

SEQ ID NO: 60 - protein, 32 aa, Artificial
  FR-H3
RVTITADESTSTAYMELSSLRSEDTAVYYCAR

SEQ ID NO: 61 - protein, 11 aa, Artificial
  FR-H4
WGQGTLVTVSS